European Patent Specification EP 3 837 378 B1, published April 5, 2023. Title: APTAMER BARCODING. Applicant: Cellular Research, Inc. Chang, Christina Shum, Eleen Li, Sixing Nakamoto, Margaret. The sequence listing filed with the application follows.

SEQUENCE LISTING (8 sequences)

SEQ ID NO: 1 - DNA, 20 bp, Artificial Sequence
  note="Description of Artificial Sequence: Synthetic Oligonucleotide"
aaaaaaaaaaaaaaaaaaaa

SEQ ID NO: 2 - DNA, 20 bp, Artificial Sequence
  note="Description of Artificial Sequence: Synthetic Oligonucleotide"
tttttttttttttttttttt

SEQ ID NO: 3 - DNA, 95 bp, Artificial Sequence
  note="Description of Artificial Sequence: Synthetic Oligonucleotide"
  5AmMC6 (1)..(1): 5' Amino Modifier C6
gttgtcaagatgctaccgttcagagtacgtggagttggtggcccgaccccgagcgctacgagccccccggaaaaaaaaaaaaaaaaaaaaaaaaa

SEQ ID NO: 4 - DNA, 200 bp, Artificial Sequence
  note="Description of Artificial Sequence: Synthetic Oligonucleotide"
  5AmMC6 (1)..(1): 5' Amino Modifier C6
gttgtcaagatgctaccgttcagagctactgtccgaagttaccgtgtatctaccacgggtggtttttcgaatccggaaaagatagtaataagtgttttagttggaataagtcgcaacttttggagacggttacctctcaatttttctgatccgtaggccccccgatctcggcctcaaaaaaaaaaaaaaaaaaaaaaaaa

SEQ ID NO: 5 - DNA, 25 bp, Artificial Sequence
  note="Description of Artificial Sequence: Synthetic Oligonucleotide"
gttgtcaagatgctaccgttcagag

SEQ ID NO: 6 - DNA, 20 bp, Artificial Sequence
  note="Description of Artificial Sequence: Synthetic Oligonucleotide"
acacgacgctcttccgatct

SEQ ID NO: 7 - DNA, 95 bp, Artificial Sequence
  note="Description of Artificial Sequence: Synthetic Oligonucleotide"
gttgtcaagatgctaccgttcagagccccatgtctagtacctattggtcccctatcctcagattcgtttaaaaaaaaaaaaaaaaaaaaaaaaaa

SEQ ID NO: 8 - DNA, 26 bp, Artificial Sequence
  note="Description of Artificial Sequence: Synthetic Oligonucleotide"
tttttttttttttttttttttttttt